European Patent Specification EP 3 568 492 B1, published January 1, 2025. Title: MULTIPLEXED SIGNAL AMPLIFICATION. Applicant: PRESIDENT AND FELLOWS OF HARVARD COLLEGE. Application Not Yet Assigned. The sequence listing filed with the application follows.

SEQUENCE LISTING (42 sequences)

SEQ ID NO: 1 - DNA, 10 bp, Artificial sequence
  Synthetic polynucleotide
  misc_feature (1)..(1): modified by /5Cy5/
ttctcttatt

SEQ ID NO: 2 - DNA, 43 bp, Artificial sequence
  Synthetic polynucleotide
  misc_feature (43)..(43): modified by /3InvdT/
actaaattcagggccttttggccctgaatttagtaataagaga

SEQ ID NO: 3 - DNA, 43 bp, Artificial sequence
  Synthetic polynucleotide
  misc_feature (43)..(43): modified by /3InvdT/
atatcccatagggccttttggccctatgggatattgaatttag

SEQ ID NO: 4 - DNA, 43 bp, Artificial sequence
  Synthetic polynucleotide
  misc_feature (43)..(43): modified by /3InvdT/
attacactacgggccttttggcccgtagtgtaattatgggata

SEQ ID NO: 5 - DNA, 43 bp, Artificial sequence
  Synthetic polynucleotide
  misc_feature (43)..(43): modified by /3InvdT/
atattaaaccgggccttttggcccggtttaatatgtagtgtaa

SEQ ID NO: 6 - DNA, 43 bp, Artificial sequence
  Synthetic polynucleotide
  misc_feature (43)..(43): modified by /3InvdT/
atcatttttcgggccttttggcccgaaaaatgatggtttaata

SEQ ID NO: 7 - DNA, 43 bp, Artificial sequence
  Synthetic polynucleotide
  misc_feature (43)..(43): modified by /3InvdT/
atctcttattgggccttttggcccaataagagataataagaga

SEQ ID NO: 8 - DNA, 22 bp, Artificial sequence
  Synthetic polynucleotide
  misc_feature (1)..(1): modified by /5ATTO565N/
  misc_feature (22)..(22): modified by /3InvdT/
ttaataagagataataagagat

SEQ ID NO: 9 - DNA, 55 bp, Artificial sequence
  Synthetic polynucleotide
ccactgtaggacgtggaatatggcaagaaaactgaaaatcatggttcatcatcat

SEQ ID NO: 10 - DNA, 43 bp, Artificial sequence
  Synthetic polynucleotide
  misc_feature (43)..(43): modified by /3InvdT/
acatcatcatgggccttttggcccatgatgatgtatgatgatg

SEQ ID NO: 11 - DNA, 43 bp, Artificial sequence
  Synthetic polynucleotide
  misc_feature (43)..(43): modified by /3InvdT/
accaataatagggccttttggccctattattggttattattgg

SEQ ID NO: 12 - DNA, 39 bp, Artificial sequence
  Synthetic polynucleotide
ctagatcgaactattcgaacactaaatattccaataata

SEQ ID NO: 13 - DNA, 28 bp, Artificial sequence
  Synthetic polynucleotide
  misc_feature (1)..(1): modified by /5ThioMC6-D/
tatttagtgttcgaatagttcgatctag

SEQ ID NO: 14 - DNA, 22 bp, Artificial sequence
  Synthetic polynucleotide
  misc_feature (1)..(1): modified by /5Alex647N/
  misc_feature (22)..(22): modified by /3InvdT/
tttattattggttattattggt

SEQ ID NO: 15 - DNA, 53 bp, Artificial sequence
  Synthetic polynucleotide
agatgagtgagttacactgaaaaacacattcgttggaaacggtttctcttatt

SEQ ID NO: 16 - DNA, 55 bp, Artificial sequence
  Synthetic polynucleotide
ccactgtaggacgtggaatatggcaagaaaactgaaaatcatggttttacactac

SEQ ID NO: 17 - DNA, 43 bp, Artificial sequence; identical to SEQ ID NO: 7
  Synthetic polynucleotide
  misc_feature (43)..(43): modified by /3InvdT/

SEQ ID NO: 18 - DNA, 43 bp, Artificial sequence
  Synthetic polynucleotide
  misc_feature (43)..(43): modified by /3InvdT/
attacactacgggccttttggcccgtagtgtaatgtagtgtaa

SEQ ID NO: 19 - DNA, 32 bp, Artificial sequence
  Synthetic polynucleotide
  misc_feature (1)..(1): modified by /5Alex647N/
  misc_feature (32)..(32): modified by /3InvdT/
ttaataagagataataagagataataagagat

SEQ ID NO: 20 - DNA, 32 bp, Artificial sequence
  Synthetic polynucleotide
  misc_feature (1)..(1): modified by /5ATTO565N/
  misc_feature (32)..(32): modified by /3InvdT/
ttgtagtgtaatgtagtgtaatgtagtgtaat

SEQ ID NO: 21 - DNA, 60 bp, Artificial sequence
  Synthetic polynucleotide
ctagatcgaactattcgaacactaaatattacatcatcatacatcatcatacaacttaac

SEQ ID NO: 22 - DNA, 43 bp, Artificial sequence
  Synthetic polynucleotide
  misc_feature (43)..(43): modified by /3InvdT/
acaacttaacgggccttttggcccgttaagttgtgttaagttg

SEQ ID NO: 23 - DNA, 28 bp, Artificial sequence
  Synthetic polynucleotide
  misc_feature (1)..(1): modified by /5ThioMC6-D/
tatttagtgttcgaatagttcgatctag

SEQ ID NO: 24 - DNA, 28 bp, Artificial sequence
  Synthetic polynucleotide
  misc_feature (1)..(1): modified by /5ThioMC6-D/
tatttagtgttcgaatagttcgatctag

SEQ ID NO: 25 - DNA, 60 bp, Artificial sequence; identical to SEQ ID NO: 21
  Synthetic polynucleotide

SEQ ID NO: 26 - DNA, 43 bp, Artificial sequence; identical to SEQ ID NO: 22
  Synthetic polynucleotide
  misc_feature (43)..(43): modified by /3InvdT/

SEQ ID NO: 27 - DNA, 61 bp, Artificial sequence
  Synthetic polynucleotide
gttaagttgtgttaagttgtgttaagttgtaaatactctcaaatactctcttccaataata

SEQ ID NO: 28 - DNA, 43 bp, Artificial sequence; identical to SEQ ID NO: 11
  Synthetic polynucleotide
  misc_feature (43)..(43): modified by /3InvdT/

SEQ ID NO: 29 - DNA, 22 bp, Artificial sequence
  Synthetic polynucleotide
  misc_feature (1)..(1): modified by /5Alex647N/
  misc_feature (22)..(22): modified by /3InvdT/
ttgagagtatttgagagtattt

SEQ ID NO: 30 - DNA, 22 bp, Artificial sequence
  Synthetic polynucleotide
  misc_feature (1)..(1): modified by /5Alex647N/
  misc_feature (22)..(22): modified by /3InvdT/
tttattattggttattattggt

SEQ ID NO: 31 - DNA, 42 bp, Artificial sequence
  Synthetic polynucleotide
  misc_feature (1)..(1): modified by /5ThioMC6/
aattctatgacaccgccacgccctatatcctcgcaataaccc

SEQ ID NO: 32 - DNA, 60 bp, Artificial sequence
  Synthetic polynucleotide
  misc_feature (1)..(1): modified by /5ATTO565N/
tttgggttattgcgaggatatagggcgtggcggtgtcatagaattttttttaatactctc

SEQ ID NO: 33 - DNA, 43 bp, Artificial sequence
  Synthetic polynucleotide
  misc_feature (43)..(43): modified by /3InvdT/
aaatactctcgggccttttggcccgagagtatttgagagtatt

SEQ ID NO: 34 - DNA, 41 bp, Artificial sequence
  Synthetic polynucleotide
gagagtatttgagagtatttgagagtatttttccttctatt

SEQ ID NO: 35 - DNA, 43 bp, Artificial sequence
  Synthetic polynucleotide
  misc_feature (43)..(43): modified by /3InvdT/
accttctattgggccttttggcccaatagaaggtaatagaagg

SEQ ID NO: 36 - DNA, 22 bp, Artificial sequence
  Synthetic polynucleotide
  misc_feature (1)..(1): modified by /5ATTO565N/
  misc_feature (22)..(22): modified by /3InvdT/
ttaatagaaggtaatagaaggt

SEQ ID NO: 37 - DNA, 39 bp, Artificial sequence
  Synthetic polynucleotide
ctagatcgaactattcgaacactaaatattcatcatcat

SEQ ID NO: 38 - DNA, 43 bp, Artificial sequence; identical to SEQ ID NO: 10
  Synthetic polynucleotide
  misc_feature (43)..(43): modified by /3InvdT/

SEQ ID NO: 39 - DNA, 28 bp, Artificial sequence
  Synthetic polynucleotide
  misc_feature (1)..(1): modified by /5ThioMC6-D/
tatttagtgttcgaatagttcgatctag

SEQ ID NO: 40 - DNA, 22 bp, Artificial sequence
  Synthetic polynucleotide
  misc_feature (1)..(1): modified by /5Alex647N/
  misc_feature (22)..(22): modified by /3InvdT/
ttatgatgatgtatgatgatgt

SEQ ID NO: 41 - DNA, 33 bp, Artificial Sequence
  Synthetic polynucleotide
  misc_feature (1)..(1): modified by /5ATTO488N/
ttgcgaggaaaactgaaaaaggtttctcttatt

SEQ ID NO: 42 - DNA, 22 bp, Artificial Sequence
  Synthetic polynucleotide
  misc_feature (1)..(1): modified by /5ATTO565N/
  misc_feature (22)..(22): modified by /3InvdT/
ttgagagtatttgagagtattt